European Patent Application EP 4 357 362 A1, published April 24, 2024. Title: Bispecific antibody combination and use thereof. Applicant: HARBOUR BIOMED (SHANGHAI) CO., LTD. The sequence listing filed with the application follows.

SEQUENCE LISTING (124 sequences)

SEQ ID NO: 1 - protein, 25 aa, Artificial Sequence [sequence omitted]

SEQ ID NO: 2 - protein, 25 aa, Artificial Sequence
  PR001838/PR001848/PR004469 HFWR1
EVQLLESGGGLVQPGGSLRLSCAAS

SEQ ID NO: 3 - protein, 25 aa, Artificial Sequence
  PR002408 HFWR1
QVQLVESGGGVVQPGRSLRLSCAAS

SEQ ID NO: 4 - protein, 25 aa, Artificial Sequence
  PR002410/PR003366 HFWR1
QVQLVQSGAEVKKPGSSMRVSCKAS

SEQ ID NO: 5 - protein, 25 aa, Artificial Sequence
  PR003886 HFWR1
EVQLVESGGGLVQPGGSLKLSCAAS

SEQ ID NO: 6 - protein, 7 aa, Artificial Sequence
  PR000210 HCDR1
GFNIKDT

SEQ ID NO: 7 - protein, 7 aa, Artificial Sequence
  PR001838/PR004469 HCDR1
GFTFSNY

SEQ ID NO: 8 - protein, 7 aa, Artificial Sequence
  PR001848/PR003886 HCDR1
GFTFSTY

SEQ ID NO: 9 - protein, 7 aa, Artificial Sequence
  PR002408 HCDR1
GFTFRSF

SEQ ID NO: 10 - protein, 7 aa, Artificial Sequence
  PR002410/PR003366 HCDR1
EDTFSSY

SEQ ID NO: 11 - protein, 19 aa, Artificial Sequence
  PR000210 HFWR2
YIHWVRQAPGKGLEWVARI

SEQ ID NO: 12 - protein, 19 aa, Artificial Sequence
  PR001838/PR004469 HFWR2
AMSWFRQPPETGLKWVSSI

SEQ ID NO: 13 - protein, 19 aa, Artificial Sequence
  PR001848 HFWR2
AMNWVRQAPGKGLEWVSRI

SEQ ID NO: 14 - protein, 19 aa, Artificial Sequence
  PR002408 HFWR2
GMHWVRQAPGKGLEWVAVI

SEQ ID NO: 15 - protein, 19 aa, Artificial Sequence
  PR002410/PR003366 HFWR2
AISWVRQAPGQGLEWMGGT

SEQ ID NO: 16 - protein, 19 aa, Artificial Sequence
  PR003886 HFWR2
AMNWVRQASGKGLEWVGRI

SEQ ID NO: 17 - protein, 6 aa, Artificial Sequence
  PR000210 HCDR2
YPTNGY

SEQ ID NO: 18 - protein, 6 aa, Artificial Sequence
  PR001838 HCDR2
DGSGGD

SEQ ID NO: 19 - protein, 8 aa, Artificial Sequence
  PR001848/PR003886 HCDR2
RSKYNNYA

SEQ ID NO: 20 - protein, 6 aa, Artificial Sequence
  PR002408 HCDR2
SYDASN

SEQ ID NO: 21 - protein, 6 aa, Artificial Sequence
  PR002410/PR003366 HCDR2
APIFGT

SEQ ID NO: 22 - protein, 6 aa, Artificial Sequence
  PR004469 HCDR2
DASGGD

SEQ ID NO: 23 - protein, 41 aa, Artificial Sequence
  PR000210 HFWR3
TRYADSVKGRFTISADTSKNTAYLQMNSLRAEDTAVYYCSR

SEQ ID NO: 24 - protein, 41 aa, Artificial Sequence
  PR001838/PR004469 HFWR3
TYYADSVKGRFTISRDNSKNTLYLQMNSLRAEDTAVYYCAK

SEQ ID NO: 25 - protein, 41 aa, Artificial Sequence
  PR001848 HFWR3
TYYADSVKDRFTISRDDSKSTLYLQMNSLRAEDTAVYYCVR

SEQ ID NO: 26 - protein, 41 aa, Artificial Sequence
  PR002408 HFWR3
EYYADSVKGRFIISRDNSKDTLYLQMNSLRAGDTAVYYCAK

SEQ ID NO: 27 - protein, 41 aa, Artificial Sequence
  PR002410/PR003366 HFWR3
TNYAQKFQGRVTITADKSTSTAYMELSSLRSEDTAVYYCAR

SEQ ID NO: 28 - protein, 41 aa, Artificial Sequence
  PR003886 HFWR3
TYYADSVKDRFTISRDDSKNTAYLQMNSLKTEDTAVYYCTR

SEQ ID NO: 29 - protein, 11 aa, Artificial Sequence
  PR000210 HCDR3
WGGDGFYAMDY

SEQ ID NO: 30 - protein, 15 aa, Artificial Sequence
  PR001838/PR004469 HCDR3
EGSHGTDDSHYDVDV

SEQ ID NO: 31 - protein, 14 aa, Artificial Sequence
  PR001848/PR003886 HCDR3
HGNFGNSYVSWFAY

SEQ ID NO: 32 - protein, 10 aa, Artificial Sequence
  PR002408 HCDR3
GGGLRWYFAY

SEQ ID NO: 33 - protein, 7 aa, Artificial Sequence
  PR002410/PR003366 HCDR3
GGPYFDY

SEQ ID NO: 34 - protein, 11 aa, Artificial Sequence
  PR000210/PR001848/PR002408/PR002410/PR003366/PR003886 HFWR4
WGQGTLVTVSS

SEQ ID NO: 35 - protein, 11 aa, Artificial Sequence
  PR001838/PR004469/PR007168 HFWR4
WGQGTTVTVSS

SEQ ID NO: 36 - protein, 23 aa, Artificial Sequence
  PR000210 LFWR1
DIQMTQSPSSLSASVGDRVTITC

SEQ ID NO: 37 - protein, 22 aa, Artificial Sequence
  PR001848/PR003886 LFWR1
QAVVTQEPSLTVSPGGTVTLTC

SEQ ID NO: 38 - protein, 23 aa, Artificial Sequence
  PR002408 LFWR1
EIVMTQSPATLSVSPGERATLSC

SEQ ID NO: 39 - protein, 23 aa, Artificial Sequence
  PR002410/PR003366 LFWR1
EIVMTQSPASLSVSPGERATLSC

SEQ ID NO: 40 - protein, 11 aa, Artificial Sequence
  PR000210 LCDR1
RASQDVNTAVA

SEQ ID NO: 41 - protein, 14 aa, Artificial Sequence
  PR001848/PR003886 LCDR1
RSSTGAVTTSNYAN

SEQ ID NO: 42 - protein, 11 aa, Artificial Sequence
  PR002408 LCDR1
RASQSISSNLG

SEQ ID NO: 43 - protein, 11 aa, Artificial Sequence
  PR002410/PR003366 LCDR1
RASQSVSSNLA

SEQ ID NO: 44 - protein, 15 aa, Artificial Sequence
  PR000210 LFWR2
WYQQKPGKAPKLLIY

SEQ ID NO: 45 - protein, 15 aa, Artificial Sequence
  PR001848/PR003886 LFWR2
WVQQKPGQAPRGLIG

SEQ ID NO: 46 - protein, 15 aa, Artificial Sequence
  PR002408/PR002410/PR003366 LFWR2
WYQQKPGQAPRLLIY

SEQ ID NO: 47 - protein, 7 aa, Artificial Sequence
  PR000210 LCDR2
SASFLYS

SEQ ID NO: 48 - protein, 7 aa, Artificial Sequence
  PR001848/PR003886 LCDR2
GTNKRAP

SEQ ID NO: 49 - protein, 7 aa, Artificial Sequence
  PR002408/PR002410/PR003366 LCDR2
GASTRAT

SEQ ID NO: 50 - protein, 32 aa, Artificial Sequence
  PR000210 LFWR3
GVPSRFSGSRSGTDFTLTISSLQPEDFATYYC

SEQ ID NO: 51 - protein, 32 aa, Artificial Sequence
  PR001848/PR003886 LFWR3
WTPARFSGSLLGDKAALTLLGAQPEDEAEYFC

SEQ ID NO: 52 - protein, 32 aa, Artificial Sequence
  PR002408 LFWR3
GIPARFSGSGSGTEFTLTISSLQSEDFAVYYC

SEQ ID NO: 53 - protein, 32 aa, Artificial Sequence
  PR002410/PR003366 LFWR3
GIPARVSGGGSGTEFTLTISSLQSEDFAVYYC

SEQ ID NO: 54 - protein, 9 aa, Artificial Sequence
  PR000210 LCDR3
QQHYTTPPT

SEQ ID NO: 55 - protein, 9 aa, Artificial Sequence
  PR001848/PR003886 LCDR3
ALWYSNLWV

SEQ ID NO: 56 - protein, 10 aa, Artificial Sequence
  PR002408 LCDR3
QQYQSWPPLT

SEQ ID NO: 57 - protein, 9 aa, Artificial Sequence
  PR002410/PR003366 LCDR3
QQYKNWPFT

SEQ ID NO: 58 - protein, 10 aa, Artificial Sequence
  PR000210 LFWR4
FGQGTKVEIK

SEQ ID NO: 59 - protein, 10 aa, Artificial Sequence
  PR001848/PR003886 LFWR4
FGGGTKLTVL

SEQ ID NO: 60 - protein, 10 aa, Artificial Sequence
  PR002408 LFWR4
FGGGTKVEIK

SEQ ID NO: 61 - protein, 10 aa, Artificial Sequence
  PR002410/PR003366 LFWR4
FGPGTKLEIK

SEQ ID NO: 62 - protein, 120 aa, Artificial Sequence [sequence omitted]

SEQ ID NO: 63 - protein, 124 aa, Artificial Sequence
  PR001838 VH
EVQLLESGGGLVQPGGSLRLSCAASGFTFSNYAMSWFRQPPETGLKWVSSIDGSGGDTYYADSVKGRFTISRDNSKNTLYLQMNSLRAEDTAVYYCAKEGSHGTDDSHYDVDVWGQGTTVTVSS

SEQ ID NO: 64 - protein, 125 aa, Artificial Sequence
  PR001848 VH
EVQLLESGGGLVQPGGSLRLSCAASGFTFSTYAMNWVRQAPGKGLEWVSRIRSKYNNYATYYADSVKDRFTISRDDSKSTLYLQMNSLRAEDTAVYYCVRHGNFGNSYVSWFAYWGQGTLVTVSS

SEQ ID NO: 65 - protein, 119 aa, Artificial Sequence
  PR002408 VH
QVQLVESGGGVVQPGRSLRLSCAASGFTFRSFGMHWVRQAPGKGLEWVAVISYDASNEYYADSVKGRFIISRDNSKDTLYLQMNSLRAGDTAVYYCAKGGGLRWYFAYWGQGTLVTVSS

SEQ ID NO: 66 - protein, 116 aa, Artificial Sequence
  PR002410/PR003366 VH
QVQLVQSGAEVKKPGSSMRVSCKASEDTFSSYAISWVRQAPGQGLEWMGGTAPIFGTTNYAQKFQGRVTITADKSTSTAYMELSSLRSEDTAVYYCARGGPYFDYWGQGTLVTVSS

SEQ ID NO: 67 - protein, 125 aa, Artificial Sequence
  PR003886 VH
EVQLVESGGGLVQPGGSLKLSCAASGFTFSTYAMNWVRQASGKGLEWVGRIRSKYNNYATYYADSVKDRFTISRDDSKNTAYLQMNSLKTEDTAVYYCTRHGNFGNSYVSWFAYWGQGTLVTVSS

SEQ ID NO: 68 - protein, 124 aa, Artificial Sequence
  PR004469 VH
EVQLLESGGGLVQPGGSLRLSCAASGFTFSNYAMSWFRQPPETGLKWVSSIDASGGDTYYADSVKGRFTISRDNSKNTLYLQMNSLRAEDTAVYYCAKEGSHGTDDSHYDVDVWGQGTTVTVSS

SEQ ID NO: 69 - protein, 107 aa, Artificial Sequence [sequence omitted]

SEQ ID NO: 70 - protein, 109 aa, Artificial Sequence
  PR001848/PR003886 VL
QAVVTQEPSLTVSPGGTVTLTCRSSTGAVTTSNYANWVQQKPGQAPRGLIGGTNKRAPWTPARFSGSLLGDKAALTLLGAQPEDEAEYFCALWYSNLWVFGGGTKLTVL

SEQ ID NO: 71 - protein, 108 aa, Artificial Sequence
  PR002408 VL
EIVMTQSPATLSVSPGERATLSCRASQSISSNLGWYQQKPGQAPRLLIYGASTRATGIPARFSGSGSGTEFTLTISSLQSEDFAVYYCQQYQSWPPLTFGGGTKVEIK

SEQ ID NO: 72 - protein, 107 aa, Artificial Sequence
  PR002410/PR003366 VL
EIVMTQSPASLSVSPGERATLSCRASQSVSSNLAWYQQKPGQAPRLLIYGASTRATGIPARVSGGGSGTEFTLTISSLQSEDFAVYYCQQYKNWPFTFGPGTKLEIK

SEQ ID NO: 73 - protein, 450 aa, Artificial Sequence
  PR000210 HC
EVQLVESGGGLVQPGGSLRLSCAASGFNIKDTYIHWVRQAPGKGLEWVARIYPTNGYTRYADSVKGRFTISADTSKNTAYLQMNSLRAEDTAVYYCSRWGGDGFYAMDYWGQGTLVTVSSASTKGPSVFPLAPSSKSTSGGTAALGCLVKDYFPEPVTVSWNSGALTSGVHTFPAVLQSSGLYSLSSVVTVPSSSLGTQTYICNVNHKPSNTKVDKKVEPKSCDKTHTCPPCPAPELLGGPSVFLFPPKPKDTLMISRTPEVTCVVVDVSHEDPEVKFNWYVDGVEVHNAKTKPREEQYNSTYRVVSVLTVLHQDWLNGKEYKCKVSNKALPAPIEKTISKAKGQPREPQVYTLPPSREEMTKNQVSLTCLVKGFYPSDIAVEWESNGQPENNYKTTPPVLDSDGSFFLYSKLTVDKSRWQQGNVFSCSVMHEALHNHYTQKSLSLSPGK

SEQ ID NO: 74 - protein, 356 aa, Artificial Sequence
  PR001838 HC
EVQLLESGGGLVQPGGSLRLSCAASGFTFSNYAMSWFRQPPETGLKWVSSIDGSGGDTYYADSVKGRFTISRDNSKNTLYLQMNSLRAEDTAVYYCAKEGSHGTDDSHYDVDVWGQGTTVTVSSEPKSCDKTHTCPPCPAPELLGGPSVFLFPPKPKDTLMISRTPEVTCVVVDVSHEDPEVKFNWYVDGVEVHNAKTKPREEQYNSTYRVVSVLTVLHQDWLNGKEYKCKVSNKALPAPIEKTISKAKGQPREPQVYTLPPSREEMTKNQVSLTCLVKGFYPSDIAVEWESNGQPENNYKTTPPVLDSDGSFFLYSKLTVDKSRWQQGNVFSCSVMHEALHNHYTQKSLSLSPGK

SEQ ID NO: 75 - protein, 455 aa, Artificial Sequence
  PR001848 HC
EVQLLESGGGLVQPGGSLRLSCAASGFTFSTYAMNWVRQAPGKGLEWVSRIRSKYNNYATYYADSVKDRFTISRDDSKSTLYLQMNSLRAEDTAVYYCVRHGNFGNSYVSWFAYWGQGTLVTVSSASTKGPSVFPLAPSSKSTSGGTAALGCLVKDYFPEPVTVSWNSGALTSGVHTFPAVLQSSGLYSLSSVVTVPSSSLGTQTYICNVNHKPSNTKVDKKVEPKSCDKTHTCPPCPAPEAAGGPSVFLFPPKPKDTLMISRTPEVTCVVVDVSHEDPEVKFNWYVDGVEVHNAKTKPREEQYNSTYRVVSVLTVLHQDWLNGKEYKCKVSNKALGAPIEKTISKAKGQPREPQVYTLPPSREEMTKNQVSLTCLVKGFYPSDIAVEWESNGQPENNYKTTPPVLDSDGSFFLYSKLTVDKSRWQQGNVFSCSVMHEALHNHYTQKSLSLSPGK

SEQ ID NO: 76 - protein, 449 aa, Artificial Sequence
  PR002408 HC
QVQLVESGGGVVQPGRSLRLSCAASGFTFRSFGMHWVRQAPGKGLEWVAVISYDASNEYYADSVKGRFIISRDNSKDTLYLQMNSLRAGDTAVYYCAKGGGLRWYFAYWGQGTLVTVSSASTKGPSVFPLAPSSKSTSGGTAALGCLVKDYFPEPVTVSWNSGALTSGVHTFPAVLQSSGLYSLSSVVTVPSSSLGTQTYICNVNHKPSNTKVDKKVEPKSCDKTHTCPPCPAPELLGGPSVFLFPPKPKDTLMISRTPEVTCVVVDVSHEDPEVKFNWYVDGVEVHNAKTKPREEQYNSTYRVVSVLTVLHQDWLNGKEYKCKVSNKALPAPIEKTISKAKGQPREPQVYTLPPSREEMTKNQVSLTCLVKGFYPSDIAVEWESNGQPENNYKTTPPVLDSDGSFFLYSKLTVDKSRWQQGNVFSCSVMHEALHNHYTQKSLSLSPGK

SEQ ID NO: 77 - protein, 446 aa, Artificial Sequence
  PR002408 HC
QVQLVQSGAEVKKPGSSMRVSCKASEDTFSSYAISWVRQAPGQGLEWMGGTAPIFGTTNYAQKFQGRVTITADKSTSTAYMELSSLRSEDTAVYYCARGGPYFDYWGQGTLVTVSSASTKGPSVFPLAPSSKSTSGGTAALGCLVKDYFPEPVTVSWNSGALTSGVHTFPAVLQSSGLYSLSSVVTVPSSSLGTQTYICNVNHKPSNTKVDKKVEPKSCDKTHTCPPCPAPELLGGPSVFLFPPKPKDTLMISRTPEVTCVVVDVSHEDPEVKFNWYVDGVEVHNAKTKPREEQYNSTYRVVSVLTVLHQDWLNGKEYKCKVSNKALPAPIEKTISKAKGQPREPQVYTLPPSREEMTKNQVSLTCLVKGFYPSDIAVEWESNGQPENNYKTTPPVLDSDGSFFLYSKLTVDKSRWQQGNVFSCSVMHEALHNHYTQKSLSLSPGK

SEQ ID NO: 78 - protein, 455 aa, Artificial Sequence
  PR003886 HC
EVQLVESGGGLVQPGGSLKLSCAASGFTFSTYAMNWVRQASGKGLEWVGRIRSKYNNYATYYADSVKDRFTISRDDSKNTAYLQMNSLKTEDTAVYYCTRHGNFGNSYVSWFAYWGQGTLVTVSSASTKGPSVFPLAPSSKSTSGGTAALGCLVKDYFPEPVTVSWNSGALTSGVHTFPAVLQSSGLYSLSSVVTVPSSSLGTQTYICNVNHKPSNTKVDKKVEPKSCDKTHTCPPCPAPEAAGGPSVFLFPPKPKDTLMISRTPEVTCVVVDVSHEDPEVKFNWYVDGVEVHNAKTKPREEQYNSTYRVVSVLTVLHQDWLNGKEYKCKVSNKALPAPIEKTISKAKGQPREPQVYTLPPSREEMTKNQVSLTCLVKGFYPSDIAVEWESNGQPENNYKTTPPVLDSDGSFFLYSKLTVDKSRWQQGNVFSCSVMHEALHNHYTQKSLSLSPGK

SEQ ID NO: 79 - protein, 356 aa, Artificial Sequence
  PR004469 HC
EVQLLESGGGLVQPGGSLRLSCAASGFTFSNYAMSWFRQPPETGLKWVSSIDASGGDTYYADSVKGRFTISRDNSKNTLYLQMNSLRAEDTAVYYCAKEGSHGTDDSHYDVDVWGQGTTVTVSSEPKSCDKTHTCPPCPAPELLGGPSVFLFPPKPKDTLMISRTPEVTCVVVDVSHEDPEVKFNWYVDGVEVHNAKTKPREEQYNSTYRVVSVLTVLHQDWLNGKEYKCKVSNKALPAPIEKTISKAKGQPREPQVYTLPPSREEMTKNQVSLTCLVKGFYPSDIAVEWESNGQPENNYKTTPPVLDSDGSFFLYSKLTVDKSRWQQGNVFSCSVMHEALHNHYTQKSLSLSPGK

SEQ ID NO: 80 - protein, 214 aa, Artificial Sequence
  PR004469 HC/polypeptide chain-1
DIQMTQSPSSLSASVGDRVTITCRASQDVNTAVAWYQQKPGKAPKLLIYSASFLYSGVPSRFSGSRSGTDFTLTISSLQPEDFATYYCQQHYTTPPTFGQGTKVEIKRTVAAPSVFIFPPSDEQLKSGTASVVCLLNNFYPREAKVQWKVDNALQSGNSQESVTEQDSKDSTYSLSSTLTLSKADYEKHKVYACEVTHQGLSSPVTKSFNRGEC

SEQ ID NO: 81 - protein, 215 aa, Artificial Sequence
  PR001848/PR003733/PR003886/PR003899 LC/polypeptide chain-1
QAVVTQEPSLTVSPGGTVTLTCRSSTGAVTTSNYANWVQQKPGQAPRGLIGGTNKRAPWTPARFSGSLLGDKAALTLLGAQPEDEAEYFCALWYSNLWVFGGGTKLTVLGQPKAAPSVTLFPPSSEELQANKATLVCLISDFYPGAVTVAWKADSSPVKAGVETTTPSKQSNNKYAASSYLSLTPEQWKSHRSYSCQVTHEGSTVEKTVAPTECS

SEQ ID NO: 82 - protein, 215 aa, Artificial Sequence
  PR002408/PR003338/PR004281 LC/polypeptide chain-1
EIVMTQSPATLSVSPGERATLSCRASQSISSNLGWYQQKPGQAPRLLIYGASTRATGIPARFSGSGSGTEFTLTISSLQSEDFAVYYCQQYQSWPPLTFGGGTKVEIKRTVAAPSVFIFPPSDEQLKSGTASVVCLLNNFYPREAKVQWKVDNALQSGNSQESVTEQDSKDSTYSLSSTLTLSKADYEKHKVYACEVTHQGLSSPVTKSFNRGEC

SEQ ID NO: 83 - protein, 214 aa, Artificial Sequence
  PR002410/PR004359 LC/polypeptide chain-1
EIVMTQSPASLSVSPGERATLSCRASQSVSSNLAWYQQKPGQAPRLLIYGASTRATGIPARVSGGGSGTEFTLTISSLQSEDFAVYYCQQYKNWPFTFGPGTKLEIKRTVAAPSVFIFPPSDEQLKSGTASVVCLLNNFYPREAKVQWKVDNALQSGNSQESVTEQDSKDSTYSLSSTLTLSKADYEKHKVYACEVTHQGLSSPVTKSFNRGEC

SEQ ID NO: 84 - protein, 590 aa, Artificial Sequence
  PR002828 polypeptide chain-2
EVQLVESGGGLVQPGGSLRLSCAASGFNIKDTYIHWVRQAPGKGLEWVARIYPTNGYTRYADSVKGRFTISADTSKNTAYLQMNSLRAEDTAVYYCSRWGGDGFYAMDYWGQGTLVTVSSASTKGPSVFPLAPSSKSTSGGTAALGCLVKDYFPEPVTVSWNSGALTSGVHTFPAVLQSSGLYSLSSVVTVPSSSLGTQTYICNVNHKPSNTKVDKKVEPKSCDKTHTCPPCPAPEAAGGPSVFLFPPKPKDTLMISRTPEVTCVVVDVSHEDPEVKFNWYVDGVEVHNAKTKPREEQYNSTYRVVSVLTVLHQDWLNGKEYKCKVSNKALGAPIEKTISKAKGQPREPQVYTLPPSREEMTKNQVSLTCLVKGFYPSDIAVEWESNGQPENNYKTTPPVLDSDGSFFLYSKLTVDKSRWQQGNVFSCSVMHEALHNHYTQKSLSLSPGEPKSSDKTHTPPPPPRTEVQLLESGGGLVQPGGSLRLSCAASGFTFSNYAMSWFRQPPETGLKWVSSIDGSGGDTYYADSVKGRFTISRDNSKNTLYLQMNSLRAEDTAVYYCAKEGSHGTDDSHYDVDVWGQGTTVTVSS

SEQ ID NO: 85 - protein, 589 aa, Artificial Sequence
  PR003338 polypeptide chain-2
QVQLVESGGGVVQPGRSLRLSCAASGFTFRSFGMHWVRQAPGKGLEWVAVISYDASNEYYADSVKGRFIISRDNSKDTLYLQMNSLRAGDTAVYYCAKGGGLRWYFAYWGQGTLVTVSSASTKGPSVFPLAPSSKSTSGGTAALGCLVKDYFPEPVTVSWNSGALTSGVHTFPAVLQSSGLYSLSSVVTVPSSSLGTQTYICNVNHKPSNTKVDKKVEPKSCDKTHTCPPCPAPEAAGGPSVFLFPPKPKDTLMISRTPEVTCVVVDVSHEDPEVKFNWYVDGVEVHNAKTKPREEQYNSTYRVVSVLTVLHQDWLNGKEYKCKVSNKALPAPIEKTISKAKGQPREPQVYTLPPSREEMTKNQVSLTCLVKGFYPSDIAVEWESNGQPENNYKTTPPVLDSDGSFFLYSKLTVDKSRWQQGNVFSCSVMHEALHNHYTQKSLSLSPGEPKSSDKTHTPPPPPRTEVQLLESGGGLVQPGGSLRLSCAASGFTFSNYAMSWFRQPPETGLKWVSSIDASGGDTYYADSVKGRFTISRDNSKNTLYLQMNSLRAEDTAVYYCAKEGSHGTDDSHYDVDVWGQGTTVTVSS

SEQ ID NO: 86 - protein, 455 aa, Artificial Sequence
  PR003733 polypeptide chain-2
EVQLLESGGGLVQPGGSLRLSCAASGFTFSTYAMNWVRQAPGKGLEWVSRIRSKYNNYATYYADSVKDRFTISRDDSKSTLYLQMNSLRAEDTAVYYCVRHGNFGNSYVSWFAYWGQGTLVTVSSASTKGPSVFPLAPSSKSTSGGTAALGCLVKDYFPEPVTVSWNSGALTSGVHTFPAVLQSSGLYSLSSVVTVPSSSLGTQTYICNVNHKPSNTKVDKKVEPKSCDKTHTCPPCPAPEAAGGPSVFLFPPKPKDTLMISRTPEVTCVVVDVSHEDPEVKFNWYVDGVEVHNAKTKPREEQYNSTYRVVSVLTVLHQDWLNGKEYKCKVSNKALPAPIEKTISKAKGQPREPQVYTLPPCREEMTKNQVSLWCLVKGFYPSDIAVEWESNGQPENNYKTTPPVLDSDGSFFLYSKLTVDKSRWQQGNVFSCSVMHEALHNHYTQKSLSLSPGK

SEQ ID NO: 87 - protein, 477 aa, Artificial Sequence
  PR003733/PR003899 polypeptide chain-3
EIVMTQSPASLSVSPGERATLSCRASQSVSSNLAWYQQKPGQAPRLLIYGASTRATGIPARVSGGGSGTEFTLTISSLQSEDFAVYYCQQYKNWPFTFGPGTKLEIKGGGGSGGGGSGGGGSGGGGSQVQLVQSGAEVKKPGSSMRVSCKASEDTFSSYAISWVRQAPGQGLEWMGGTAPIFGTTNYAQKFQGRVTITADKSTSTAYMELSSLRSEDTAVYYCARGGPYFDYWGQGTLVTVSSASEPKSSDKTHTCPPCPAPEAAGGPSVFLFPPKPKDTLMISRTPEVTCVVVDVSHEDPEVKFNWYVDGVEVHNAKTKPREEQYNSTYRVVSVLTVLHQDWLNGKEYKCKVSNKALPAPIEKTISKAKGQPREPQVCTLPPSREEMTKNQVSLSCAVKGFYPSDIAVEWESNGQPENNYKTTPPVLDSDGSFFLVSKLTVDKSRWQQGNVFSCSVMHEALHNHYTQKSLSLSPGK

SEQ ID NO: 88 - protein, 455 aa, Artificial Sequence
  PR003899 polypeptide chain-2
EVQLVESGGGLVQPGGSLKLSCAASGFTFSTYAMNWVRQASGKGLEWVGRIRSKYNNYATYYADSVKDRFTISRDDSKNTAYLQMNSLKTEDTAVYYCTRHGNFGNSYVSWFAYWGQGTLVTVSSASTKGPSVFPLAPSSKSTSGGTAALGCLVKDYFPEPVTVSWNSGALTSGVHTFPAVLQSSGLYSLSSVVTVPSSSLGTQTYICNVNHKPSNTKVDKKVEPKSCDKTHTCPPCPAPEAAGGPSVFLFPPKPKDTLMISRTPEVTCVVVDVSHEDPEVKFNWYVDGVEVHNAKTKPREEQYNSTYRVVSVLTVLHQDWLNGKEYKCKVSNKALPAPIEKTISKAKGQPREPQVYTLPPCREEMTKNQVSLWCLVKGFYPSDIAVEWESNGQPENNYKTTPPVLDSDGSFFLYSKLTVDKSRWQQGNVFSCSVMHEALHNHYTQKSLSLSPGK

SEQ ID NO: 89 - protein, 572 aa, Artificial Sequence
  PR004281 polypeptide chain-2
QVQLVESGGGVVQPGRSLRLSCAASGFTFRSFGMHWVRQAPGKGLEWVAVISYDASNEYYADSVKGRFIISRDNSKDTLYLQMNSLRAGDTAVYYCAKGGGLRWYFAYWGQGTLVTVSSASTKGPSVFPLAPSSKSTSGGTAALGCLVKDYFPEPVTVSWNSGALTSGVHTFPAVLQSSGLYSLSSVVTVPSSSLGTQTYICNVNHKPSNTKVDKKVEPKSCDKTHTCPPCPAPEAAGGPSVFLFPPKPKDTLMISRTPEVTCVVVDVSHEDPEVKFNWYVDGVEVHNAKTKPREEQYNSTYRVVSVLTVLHQDWLNGKEYKCKVSNKALPAPIEKTISKAKGQPREPQVYTLPPSREEMTKNQVSLTCLVKGFYPSDIAVEWESNGQPENNYKTTPPVLDSDGSFFLYSKLTVDKSRWQQGNVFSCSVMHEALHNHYTQKSLSLSPGEVQLLESGGGLVQPGGSLRLSCAASGFTFSNYAMSWFRQPPETGLKWVSSIDASGGDTYYADSVKGRFTISRDNSKNTLYLQMNSLRAEDTAVYYCAKEGSHGTDDSHYDVDVWGQGTTVTVSS

SEQ ID NO: 90 - protein, 578 aa, Artificial Sequence
  PR004282 polypeptide chain-2
QVQLVESGGGVVQPGRSLRLSCAASGFTFRSFGMHWVRQAPGKGLEWVAVISYDASNEYYADSVKGRFIISRDNSKDTLYLQMNSLRAGDTAVYYCAKGGGLRWYFAYWGQGTLVTVSSASTKGPSVFPLAPSSKSTSGGTAALGCLVKDYFPEPVTVSWNSGALTSGVHTFPAVLQSSGLYSLSSVVTVPSSSLGTQTYICNVNHKPSNTKVDKKVEPKSCDKTHTCPPCPAPEAAGGPSVFLFPPKPKDTLMISRTPEVTCVVVDVSHEDPEVKFNWYVDGVEVHNAKTKPREEQYNSTYRVVSVLTVLHQDWLNGKEYKCKVSNKALPAPIEKTISKAKGQPREPQVYTLPPSREEMTKNQVSLTCLVKGFYPSDIAVEWESNGQPENNYKTTPPVLDSDGSFFLYSKLTVDKSRWQQGNVFSCSVMHEALHNHYTQKSLSLSPGGGSGGSEVQLLESGGGLVQPGGSLRLSCAASGFTFSNYAMSWFRQPPETGLKWVSSIDASGGDTYYADSVKGRFTISRDNSKNTLYLQMNSLRAEDTAVYYCAKEGSHGTDDSHYDVDVWGQGTTVTVSS

SEQ ID NO: 91 - protein, 586 aa, Artificial Sequence
  PR004359 polypeptide chain-2
QVQLVQSGAEVKKPGSSMRVSCKASEDTFSSYAISWVRQAPGQGLEWMGGTAPIFGTTNYAQKFQGRVTITADKSTSTAYMELSSLRSEDTAVYYCARGGPYFDYWGQGTLVTVSSASTKGPSVFPLAPSSKSTSGGTAALGCLVKDYFPEPVTVSWNSGALTSGVHTFPAVLQSSGLYSLSSVVTVPSSSLGTQTYICNVNHKPSNTKVDKKVEPKSCDKTHTCPPCPAPEAAGGPSVFLFPPKPKDTLMISRTPEVTCVVVDVSHEDPEVKFNWYVDGVEVHNAKTKPREEQYNSTYRVVSVLTVLHQDWLNGKEYKCKVSNKALPAPIEKTISKAKGQPREPQVYTLPPSREEMTKNQVSLTCLVKGFYPSDIAVEWESNGQPENNYKTTPPVLDSDGSFFLYSKLTVDKSRWQQGNVFSCSVMHEALHNHYTQKSLSLSPGEPKSSDKTHTPPPPPRTEVQLLESGGGLVQPGGSLRLSCAASGFTFSNYAMSWFRQPPETGLKWVSSIDGSGGDTYYADSVKGRFTISRDNSKNTLYLQMNSLRAEDTAVYYCAKEGSHGTDDSHYDVDVWGQGTTVTVSS

SEQ ID NO: 92 - protein, 480 aa, Artificial Sequence
  PR003366 SCFV
EIVMTQSPASLSVSPGERATLSCRASQSVSSNLAWYQQKPGQAPRLLIYGASTRATGIPARVSGGGSGTEFTLTISSLQSEDFAVYYCQQYKNWPFTFGPGTKLEIKGGGGSGGGGSGGGGSGGGGSQVQLVQSGAEVKKPGSSMRVSCKASEDTFSSYAISWVRQAPGQGLEWMGGTAPIFGTTNYAQKFQGRVTITADKSTSTAYMELSSLRSEDTAVYYCARGGPYFDYWGQGTLVTVSSGGGASEPKSCDKTHTCPPCPAPELLGGPSVFLFPPKPKDTLMISRTPEVTCVVVDVSHEDPEVKFNWYVDGVEVHNAKTKPREEQYNSTYRVVSVLTVLHQDWLNGKEYKCKVSNKALPAPIEKTISKAKGQPREPQVYTLPPSREEMTKNQVSLTCLVKGFYPSDIAVEWESNGQPENNYKTTPPVLDSDGSFFLYSKLTVDKSRWQQGNVFSCSVMHEALHNHYTQKSLSLSPGK

SEQ ID NO: 93 - protein, 6 aa, Artificial Sequence
  linker peptide GS_6
GGSGGS

SEQ ID NO: 94 - protein, 20 aa, Artificial Sequence
  linker peptide GS_20
GGGGSGGGGSGGGGSGGGGS

SEQ ID NO: 95 - protein, 17 aa, Artificial Sequence
  linker peptide H1_15-RT
EPKSSDKTHTPPPPPRT

SEQ ID NO: 96 - protein, 18 aa, Artificial Sequence
  linker peptide L-H1_15-RT
LEPKSSDKTHTPPPPPRT

SEQ ID NO: 97 - protein, 7 aa, Artificial Sequence
  PR006004/PR007440/PR007168 HCDR1
GFAFSNY

SEQ ID NO: 98 - protein, 6 aa, Artificial Sequence
  PR006004 HCDR2
SGDGRS

SEQ ID NO: 99 - protein, 13 aa, Artificial Sequence
  PR007440/PR006004/PR007168 HCDR3
DRFGDDYYYGMNV

SEQ ID NO: 100 - protein, 7 aa, Artificial Sequence
  PR006008/PR007441/PR007078/PR007168 HCDR1
GFTFTDF

SEQ ID NO: 101 - protein, 6 aa, Artificial Sequence
  PR006008 HCDR2
SPDGSS

SEQ ID NO: 102 - protein, 13 aa, Artificial Sequence
  PR006008/PR007441/PR007078/PR007168 HCDR3
FSTGWHRIEYFQH

SEQ ID NO: 103 - protein, 6 aa, Artificial Sequence
  PR007440/PR007168 HCDR2
SGDSRS

SEQ ID NO: 104 - protein, 6 aa, Artificial Sequence
  PR007441/PR007078/PR007168 HCDR2
SPDSSS

SEQ ID NO: 105 - protein, 354 aa, Artificial Sequence
  PR006004 heavy chain
EVQLVESGGGLVQPGGSLRLSCAASGFAFSNYWMHWARQVPGKGRVWISRISGDGRSTSYADSVKGRFTISRDNAKNMVYLQMNNLRAEDTAVYYCARDRFGDDYYYGMNVWGQGTTVTVSSEPKSSDKTHTCPPCPAPELLGGPSVFLFPPKPKDTLMISRTPEVTCVVVDVSHEDPEVKFNWYVDGVEVHNAKTKPREEQYNSTYRVVSVLTVLHQDWLNGKEYKCKVSNKALPAPIEKTISKAKGQPREPQVYTLPPSREEMTKNQVSLTCLVKGFYPSDIAVEWESNGQPENNYKTTPPVLDSDGSFFLYSKLTVDKSRWQQGNVFSCSVMHEALHNHYTQKSLSLSPGK

SEQ ID NO: 106 - protein, 122 aa, Artificial Sequence
  PR006004 VH
EVQLVESGGGLVQPGGSLRLSCAASGFAFSNYWMHWARQVPGKGRVWISRISGDGRSTSYADSVKGRFTISRDNAKNMVYLQMNNLRAEDTAVYYCARDRFGDDYYYGMNVWGQGTTVTVSS

SEQ ID NO: 107 - protein, 354 aa, Artificial Sequence
  PR006008 heavy chain
EVQLVESGGGLVQPGGSLRLSCAASGFTFTDFWMHWVRQVPGKGREWVSRISPDGSSTSYEDSVKGRFTISRDNAKNTVYLQMHGLRAEDTAVYYCTRFSTGWHRIEYFQHWGQGTLVTVSSEPKSSDKTHTCPPCPAPELLGGPSVFLFPPKPKDTLMISRTPEVTCVVVDVSHEDPEVKFNWYVDGVEVHNAKTKPREEQYNSTYRVVSVLTVLHQDWLNGKEYKCKVSNKALPAPIEKTISKAKGQPREPQVYTLPPSREEMTKNQVSLTCLVKGFYPSDIAVEWESNGQPENNYKTTPPVLDSDGSFFLYSKLTVDKSRWQQGNVFSCSVMHEALHNHYTQKSLSLSPGK

SEQ ID NO: 108 - protein, 122 aa, Artificial Sequence
  PR006008 VH
EVQLVESGGGLVQPGGSLRLSCAASGFTFTDFWMHWVRQVPGKGREWVSRISPDGSSTSYEDSVKGRFTISRDNAKNTVYLQMHGLRAEDTAVYYCTRFSTGWHRIEYFQHWGQGTLVTVSS

SEQ ID NO: 109 - protein, 354 aa, Artificial Sequence
  PR007440 heavy chain
EVQLVESGGGLVQPGGSLRLSCAASGFAFSNYWMHWARQVPGKGRVWISRISGDSRSTSYADSVKGRFTISRDNAKNMVYLQMNNLRAEDTAVYYCARDRFGDDYYYGMNVWGQGTTVTVSSEPKSSDKTHTCPPCPAPELLGGPSVFLFPPKPKDTLMISRTPEVTCVVVDVSHEDPEVKFNWYVDGVEVHNAKTKPREEQYNSTYRVVSVLTVLHQDWLNGKEYKCKVSNKALPAPIEKTISKAKGQPREPQVYTLPPSREEMTKNQVSLTCLVKGFYPSDIAVEWESNGQPENNYKTTPPVLDSDGSFFLYSKLTVDKSRWQQGNVFSCSVMHEALHNHYTQKSLSLSPGK

SEQ ID NO: 110 - protein, 122 aa, Artificial Sequence
  PR007440 VH
EVQLVESGGGLVQPGGSLRLSCAASGFAFSNYWMHWARQVPGKGRVWISRISGDSRSTSYADSVKGRFTISRDNAKNMVYLQMNNLRAEDTAVYYCARDRFGDDYYYGMNVWGQGTTVTVSS

SEQ ID NO: 111 - protein, 354 aa, Artificial Sequence
  PR007441 heavy chain
EVQLVESGGGLVQPGGSLRLSCAASGFTFTDFWMHWVRQVPGKGREWVSRISPDSSSTSYEDSVKGRFTISRDNAKNTVYLQMHGLRAEDTAVYYCTRFSTGWHRIEYFQHWGQGTLVTVSSEPKSSDKTHTCPPCPAPELLGGPSVFLFPPKPKDTLMISRTPEVTCVVVDVSHEDPEVKFNWYVDGVEVHNAKTKPREEQYNSTYRVVSVLTVLHQDWLNGKEYKCKVSNKALPAPIEKTISKAKGQPREPQVYTLPPSREEMTKNQVSLTCLVKGFYPSDIAVEWESNGQPENNYKTTPPVLDSDGSFFLYSKLTVDKSRWQQGNVFSCSVMHEALHNHYTQKSLSLSPGK

SEQ ID NO: 112 - protein, 122 aa, Artificial Sequence
  PR007441 VH
EVQLVESGGGLVQPGGSLRLSCAASGFTFTDFWMHWVRQVPGKGREWVSRISPDSSSTSYEDSVKGRFTISRDNAKNTVYLQMHGLRAEDTAVYYCTRFSTGWHRIEYFQHWGQGTLVTVSS

SEQ ID NO: 113 - protein, 215 aa, Artificial Sequence; identical to SEQ ID NO: 81
  PR007078/PR007168 polypeptide chain-1

SEQ ID NO: 114 - protein, 455 aa, Artificial Sequence
  PR007078/PR007168 polypeptide chain-2
EVQLVESGGGLVQPGGSLKLSCAASGFTFSTYAMNWVRQASGKGLEWVGRIRSKYNNYATYYADSVKDRFTISRDDSKNTAYLQMNSLKTEDTAVYYCTRHGNFGNSYVSWFAYWGQGTLVTVSSASTKGPSVFPLAPSSKSTSGGTAALGCLVKDYFPEPVTVSWNSGALTSGVHTFPAVLQSSGLYSLSSVVTVPSSSLGTQTYICNVNHKPSNTKVDKKVEPKSCDKTHTCPPCPAPEAAGAPSVFLFPPKPKDTLMISRTPEVTCVVVDVSHEDPEVKFNWYVDGVEVHNAKTKPREEQYNSTYRVVSVLTVLHQDWLNGKEYKCKVSNKALPAPIEKTISKAKGQPREPQVYTLPPCREEMTKNQVSLWCLVKGFYPSDIAVEWESNGQPENNYKTTPPVLDSDGSFFLYSKLTVDKSRWQQGNVFSCSVMHEALHNHYTQKSLSLSPGK

SEQ ID NO: 115 - protein, 493 aa, Artificial Sequence
  PR007078 polypeptide chain-3
EVQLVESGGGLVQPGGSLRLSCAASGFTFTDFWMHWVRQVPGKGREWVCRISPDSSSTSYEDSVKGRFTCSRDNAKNTVYLQMHGLRAEDTAVYYCTRFSTGWHRIEYFQHWGQGTLVTVSSGGGGSGGGGSGGGGSEVQLVESGGGLVQPGGSLRLSCAASGFTFTDFWMHWVRQVPGKGREWVCRISPDSSSTSYEDSVKGRFTCSRDNAKNTVYLQMHGLRAEDTAVYYCTRFSTGWHRIEYFQHWGQGTLVTVSSASEPKSSDKTHTCPPCPAPEAAGAPSVFLFPPKPKDTLMISRTPEVTCVVVDVSHEDPEVKFNWYVDGVEVHNAKTKPREEQYNSTYRVVSVLTVLHQDWLNGKEYKCKVSNKALPAPIEKTISKAKGQPREPQVCTLPPSREEMTKNQVSLSCAVKGFYPSDIAVEWESNGQPENNYKTTPPVLDSDGSFFLVSKLTVDKSRWQQGNVFSCSVMHEALHNHYTQKSLSLSPGK

SEQ ID NO: 116 - protein, 493 aa, Artificial Sequence
  PR007168 polypeptide chain-3
EVQLVESGGGLVQPGGSLRLSCAASGFAFSNYWMHWARQVPGKGRVWICRISGDSRSTSYADSVKGRFTCSRDNAKNMVYLQMNNLRAEDTAVYYCARDRFGDDYYYGMNVWGQGTTVTVSSGGGGSGGGGSGGGGSEVQLVESGGGLVQPGGSLRLSCAASGFTFTDFWMHWVRQVPGKGREWVCRISPDSSSTSYEDSVKGRFTCSRDNAKNTVYLQMHGLRAEDTAVYYCTRFSTGWHRIEYFQHWGQGTLVTVSSASEPKSSDKTHTCPPCPAPEAAGAPSVFLFPPKPKDTLMISRTPEVTCVVVDVSHEDPEVKFNWYVDGVEVHNAKTKPREEQYNSTYRVVSVLTVLHQDWLNGKEYKCKVSNKALPAPIEKTISKAKGQPREPQVCTLPPSREEMTKNQVSLSCAVKGFYPSDIAVEWESNGQPENNYKTTPPVLDSDGSFFLVSKLTVDKSRWQQGNVFSCSVMHEALHNHYTQKSLSLSPGK

SEQ ID NO: 117 - protein, 19 aa, Artificial Sequence
  PR007078/PR007168 HFWR2
WMHWVRQVPGKGREWVCRI

SEQ ID NO: 118 - protein, 41 aa, Artificial Sequence
  PR007078/PR007168 HFWR3
TSYEDSVKGRFTCSRDNAKNTVYLQMHGLRAEDTAVYYCTR

SEQ ID NO: 119 - protein, 11 aa, Artificial Sequence
  PR007078/PR007168 HFWR4
WGQGTLVTVSS

SEQ ID NO: 120 - protein, 19 aa, Artificial Sequence
  PR007168 HFWR2
WMHWARQVPGKGRVWICRI

SEQ ID NO: 121 - protein, 41 aa, Artificial Sequence
  PR007168 HFWR3
TSYADSVKGRFTCSRDNAKNMVYLQMNNLRAEDTAVYYCAR

SEQ ID NO: 122 - protein, 259 aa, Artificial Sequence
  PR007078 VH_A-VH_B
EVQLVESGGGLVQPGGSLRLSCAASGFTFTDFWMHWVRQVPGKGREWVCRISPDSSSTSYEDSVKGRFTCSRDNAKNTVYLQMHGLRAEDTAVYYCTRFSTGWHRIEYFQHWGQGTLVTVSSGGGGSGGGGSGGGGSEVQLVESGGGLVQPGGSLRLSCAASGFTFTDFWMHWVRQVPGKGREWVCRISPDSSSTSYEDSVKGRFTCSRDNAKNTVYLQMHGLRAEDTAVYYCTRFSTGWHRIEYFQHWGQGTLVTVSS

SEQ ID NO: 123 - protein, 259 aa, Artificial Sequence
  PR007168 VH_A-VH_B
EVQLVESGGGLVQPGGSLRLSCAASGFTFTDFWMHWVRQVPGKGREWVCRISPDSSSTSYEDSVKGRFTCSRDNAKNTVYLQMHGLRAEDTAVYYCTRFSTGWHRIEYFQHWGQGTLVTVSSGGGGSGGGGSGGGGSEVQLVESGGGLVQPGGSLRLSCAASGFAFSNYWMHWARQVPGKGRVWICRISGDSRSTSYADSVKGRFTCSRDNAKNMVYLQMNNLRAEDTAVYYCARDRFGDDYYYGMNVWGQGTTVTVSS

SEQ ID NO: 124 - protein, 15 aa, Artificial Sequence
  linker peptide GS_15
GGGGSGGGGSGGGGS